European Patent Specification EP 3 281 939 B1, published October 18, 2023. Title: Stable Crystal of 4-Oxoquinoline Compound. Applicant: Japan Tobacco Inc. The sequence listing filed with the application follows.

SEQUENCE LISTING (4 sequences)

SEQ ID NO: 1 - DNA, 32 bp, Artificial Sequence
  Donor plus strand for activity determination of HIV integrase.
acccttttagtcagtgtggaaaatctctagca

SEQ ID NO: 2 - DNA, 31 bp, Artificial Sequence
  Donor minus strand for activity determination of HIV integrase.
actgctagagattttccacactgactaaaag

SEQ ID NO: 3 - DNA, 20 bp, Artificial Sequence
  Target plus strand for activity determination of HIV integrase.
tgaccaagggctaattcact

SEQ ID NO: 4 - DNA, 20 bp, Artificial Sequence
  Target minus strand for activity determination of HIV integrase.
agtgaattagcccttggtca